European Patent Specification EP 3 301 154 B1, published January 25, 2023. Title: Laundry Detergent Composition. Applicant: The Procter and Gamble Company. The sequence listing filed with the application follows.

SEQUENCE LISTING (14 sequences)

SEQ ID NO: 1 - protein, 269 aa, Thermomyces lanuginosus [sequence omitted]

SEQ ID NO: 2 - protein, 773 aa, Bacillus sp.
AEGNTREDNFKHLLGNDNVKRPSEAGALQLQEVDGQMTLVDQHGEKIQLRGMSTHGLQWFPEILNDNAYKALANDWESNMIRLAMYVGENGYASNPELIKSRVIKGIDLAIENDMYVIVDWHVHAPGDPRDPVYAGAEDFFRDIAALYPNNPHIIYELANEPSSNNNGGAGIPNNEEGWNAVKEYADPIVEMLRDSGNADDNIIIVGSPNWSQRPDLAADNPINDHHTMYTVHFYTGSHAASTESYPPETPNSERGNVMSNTRYALENGVAVFATEWGTSQANGDGGPYFDEADVWIEFLNENNISWANWSLTNKNEVSGAFTPFELGKSNATNLDPGPDHVWAPEELSLSGEYVRARIKGVNYEPIDRTKYTKVLWDFNDGTKQGFGVNSDSPNKELIAVDNENNTLKVSGLDVSNDVSDGNFWANARLSADGWGKSVDILGAEKLTMDVIVDEPTTVAIAAIPQSSKSGWANPERAVRVNAEDFVQQTDGKYKAGLTITGEDAPNLKNIAFHEEDNNMNNIILFVGTDAADVIYLDNIKVIGTEVEIPVVHDPKGEAVLPSVFEDGTRQGWDWAGESGVKTALTIEEANGSNALSWEFGYPEVKPSDNWATAPRLDFWKSDLVRGENDYVAFDFYLDPVRATEGAMNINLVFQPPTNGYWVQAPKTYTINFDELEEANQVNGLYHYEVKINVRDITNIQDDTLLRNMMIIFADVESDFAGRVFVDNVRFEGAATTEPVEPEPVDPGEETPPVDEKEAKKEQKEAEKEEKEE

SEQ ID NO: 3 - protein, 524 aa, Paenibacillus polymyxa
VVHGQTAKTITIKVDTFKDRKPISPYIYGTNQDLAGDENMAARRLGGNRMTGYNWENNMSNAGSDWQQSSDNYLCSNGGLTQAECEKPGAVTTSFHDQSLKLGTYSLVTLPMAGYVAKDGNGSVQESEKAPSARWNQVVNAKNAPFQLQPDLNDNRVYVDEFVHFLVNKYGTASTKAGVKGYALDNEPALWSHTHPRIHGEKVGAKELVDRSVSLSKAVKAIDAGAEVFGPVLYGFGAYKDLQTAPDWDSVKGNYSWFVDYYLDQMRLSSQVEGKRLLDVFDVHWYPEAMGGGIRITNEVGNDETKKARMQAPRTLWDPTYKEDSWIAQWNSEFLPILPRLKQSVDKYYPGTKLAMTEYSYGGENDISGGIAMTDVLGILGKNDVYMANYWKLKDGVNNYVSAAYKLYRNYDGKNSTFGDTSVSAQTSDIVNSSVHASVTNASDKELHLVVMNKSMDSAFDAQFDLSGAKTYISGKVWGFDKNSSQIKEAAPITQISGNRFTYTVPPLTAYHIVLTTGNDTSPV

SEQ ID NO: 4 - protein, 283 aa, Artificial Sequence
  Hybrid protein containing fragments originating from proteins endogenous to Melanocarpus albomyces and Trichoderma reesei
ANGQSTRYWDCCKPSCGWRGKGPVNQPVYSCDANFQRIHDFDAVSGCEGGPAFSCADHSPWAINDNLSYGFAATALSGQTEESWCCACYALTFTSGPVAGKTMVVQSTSTGGDLGSNHFDLNIPGGGVGLFDGCTPQFGGLPGARYGGISSRQECDSFPEPLKPGCQWRFDWFQNADNPSFTFERVQCPEELVARTGCRRHDDGGFPAVQIPSSTGNPSGGNPPGGNPPGTTTTRRPATTTGSSPGPTQSHYGQCGGIGYSGPTVCASGTTCQVLNPYYSQCL

SEQ ID NO: 5 - protein, 485 aa, Bacillus sp.
HHNGTNGTMMQYFEWHLPNDGNHWNRLRDDASNLRNRGITAIWIPPAWKGTSQNDVGYGAYDLYDLGEFNQKGTVRTKYGTRSQLESAIHALKNNGVQVYGDVVMNHKGGADATENVLAVEVNPNNRNQEISGDYTIEAWTKFDFPGRGNTYSDFKWRWYHFDGVDWDQSRQFQNRIYKFRGDGKAWDWEVDSENGNYDYLMYADVDMDHPEVVNELRRWGEWYTNTLNLDGFRIDAVKHIKYSFTRDWLTHVRNATGKEMFAVAEFWKNDLGALENYLNKTNWNHSVFDVPLHYNLYNASNSGGNYDMAKLLNGTVVQKHPMHAVTFVDNHDSQPGESLESFVQEWFKPLAYALILTREQGYPSVFYGDYYGIPTHSVPAMKAKIDPILEARQNFAYGTQHDYFDHHNIIGWTREGNTTHPNSGLATIMSDGPGGEKWMYVGQNKAGQVWHDITGNKPGTVTINADGWANFSVNGGSVSIWVKR

SEQ ID NO: 6 - protein, 485 aa, Bacillus sp.
HHNGTNGTMMQYFEWYLPNDGNHWNRLRSDASNLKDKGISAVWIPPAWKGASQNDVGYGAYDLYDLGEFNQKGTIRTKYGTRNQLQAAVNALKSNGIQVYGDVVMNHKGGADATEMVRAVEVNPNNRNQEVSGEYTIEAWTKFDFPGRGNTHSNFKWRWYHFDGVDWDQSRKLNNRIYKFRGDGKGWDWEVDTENGNYDYLMYADIDMDHPEVVNELRNWGVWYTNTLGLDGFRIDAVKHIKYSFTRDWINHVRSATGKNMFAVAEFWKNDLGAIENYLNKTNWNHSVFDVPLHYNLYNASKSGGNYDMRQIFNGTVVQRHPMHAVTFVDNHDSQPEEALESFVEEWFKPLAYALTLTREQGYPSVFYGDYYGIPTHGVPAMKSKIDPILEARQKYAYGRQNDYLDHHNIIGWTREGNTAHPNSGLATIMSDGAGGNKWMFVGRNKAGQVWTDITGNRAGTVTINADGWGNFSVNGGSVSIWVNK

SEQ ID NO: 7 - protein, 480 aa, Bacillus sp. KSM-K38
DGLNGTMMQYYEWHLENDGQHWNRLHDDAAALSDAGITAIWIPPAYKGNSQADVGYGAYDLYDLGEFNQKGTVRTKYGTKAQLERAIGSLKSNDINVYGDVVMNHKMGADFTEAVQAVQVNPTNRWQDISGAYTIDAWTGFDFSGRNNAYSDFKWRWFHFNGVDWDQRYQENHIFRFANTNWNWRVDEENGNYDYLLGSNIDFSHPEVQDELKDWGSWFTDELDLDGYRLDAIKHIPFWYTSDWVRHQRNEADQDLFVVGEYWKDDVGALEFYLDEMNWEMSLFDVPLNYNFYRASQQGGSYDMRNILRGSLVEAHPMHAVTFVDNHDTQPGESLESWVADWFKPLAYATILTREGGYPNVFYGDYYGIPNDNISAKKDMIDELLDARQNYAYGTQHDYFDHWDVVGWTREGSSSRPNSGLATIMSNGPGGSKWMYVGRQNAGQTWTDLTGNNGASVTINGDGWGEFFTNGGSVSVYVNQ

SEQ ID NO: 8 - protein, 483 aa, Cytophaga sp.
AATNGTMMQYFEWYVPNDGQQWNRLRTDAPYLSSVGITAVWTPPAYKGTSQADVGYGPYDLYDLGEFNQKGTVRTKYGTKGELKSAVNTLHSNGIQVYGDVVMNHKAGADYTENVTAVEVNPSNRNQETSGEYNIQAWTGFNFPGRGTTYSNFKWQWFHFDGTDWDQSRSLSRIFKFTGKAWDWPVSSENGNYDYLMYADYDYDHPDVVNEMKKWGVWYANEVGLDGYRLDAVKHIKFSFLKDWVDNARAATGKEMFTVGEYWQNDLGALNNYLAKVNYNQSLFDAPLHYNFYAASTGGGYYDMRNILNNTLVASNPTKAVTLVENHDTQPGQSLESTVQPWFKPLAYAFILTRSGGYPSVFYGDMYGTKGTTTREIPALKSKIEPLLKARKDYAYGTQRDYIDNPDVIGWTREGDSTKAKSGLATVITDGPGGSKRMYVGTSNAGEIWYDLTGNNSTKITIGSDGYATFPVNKGSVSVWVQQ

SEQ ID NO: 9 - protein, 300 aa, Bacillus amyloliquefaciens
AATTGTGTTLKGKTVSLNISSESGKYVLRDLSKPTGTQIITYDLQNREYNLPGTLVSSTTNQFTTSSQRAAVDAHYNLGKVYDYFYQKFNRNSYDNKGGKIVSSVHYGSRYNNAAWIGDQMIYGDGDGSFFSPLSGSMDVTAHEMTHGVTQETANLNYENQPGALNESFSDVFGYFNDTEDWDIGEDITVSQPALRSLSNPTKYGQPDNFKNYKNLPNTDAGDYGGVHTNSGIPNKAAYNTITKIGVNKAEQIYYRALTVYLTPSSTFKDAKAALIQSARDLYGSQDAASVEAAWNAVGL

SEQ ID NO: 10 - protein, 275 aa, Bacillus amyloliquefaciens [sequence omitted]

SEQ ID NO: 11 - protein, 316 aa, Bacillus thermoproteolyticus
ITGTSTVGVGRGVLGDQKNINTTYSTYYYLQDNTRGNGIFTYDAKYRTTLPGSLWADADNQFFASYDAPAVDAHYYAGVTYDYYKNVHNRLSYDGNNAAIRSSVHYSQGYNNAFWNGSQMVYGDGDGQTFIPLSGGIDVVAHELTHAVTDYTAGLIYQNESGAINEAISDIFGTLVEFYANKNPDWEIGEDVYTPGISGDSLRSMSDPAKYGDPDHYSKRYTGTQDNGGVHINSGIINKAAYLISQGGTHYGVSVVGIGRDKLGKIFYRALTQYLTPTSNFSQLRAAAVQSATDLYGSTSQEVASVKQAFDAVGVK

SEQ ID NO: 12 - protein, 269 aa, Bacillus lentus
AQSVPWGISRVQAPAAHNRGLTGSGVKVAVLDTGISTHPDLNIRGGASFVPGEPSTQDGNGHGTHVAGTIAALNNSIGVLGVAPSAELYAVKVLGASGSGSVSSIAQGLEWAGNNGMHVANLSLGSPSPSATLEQAVNSATSRGVLVVAASGNSGAGSISYPARYANAMAVGATDQNNNRASFSQYGAGLDIVAPGVNVQSTYPGSTYASLNGTSMATPHVAGAAALVKQKNPSWSNVQIRNHLKNTATSLGSTNLYGSGLVNAEAATR

SEQ ID NO: 13 - protein, 311 aa, Bacillus sp. TY145 [sequence omitted]

SEQ ID NO: 14 - protein, 434 aa, Bacillus sp. KSM-KP43
NDVARGIVKADVAQSSYGLYGQGQIVAVADTGLDTGRNDSSMHEAFRGKITALYALGRTNNANDTNGHGTHVAGSVLGNGSTNKGMAPQANLVFQSIMDSGGGLGGLPSNLQTLFSQAYSAGARIHTNSWGAAVNGAYTTDSRNVDDYVRKNDMTILFAAGNEGPNGGTISAPGTAKNAITVGATENLRPSFGSYADNINHVAQFSSRGPTKDGRIKPDVMAPGTFILSARSSLAPDSSFWANHDSKYAYMGGTSMATPIVAGNVAQLREHFVKNRGITPKPSLLKAALIAGAADIGLGYPNGNQGWGRVTLDKSLNVAYVNESSSLSTSQKATYSFTATAGKPLKISLVWSDAPASTTASVTLVNDLDLVITAPNGTQYVGNDFTSPYNDNWDGRNNVENVFINAPQSGTYTIEVQAYNVPVGPQTFSLAIVN